European Patent Specification EP 4 247 415 B1, published July 29, 2026. Title: Pharmaceutical composition for treating non-alcoholic fatty liver, non-alcoholic steatohepatitis, or hepatic fibrosis using Ssu72 protein or a polynucleotide encoding the same. Applicant: CUROGEN Technology Co., Ltd. Research and Business Foundation SUNGKYUNKWAN UNIVERSITY. The sequence listing filed with the application follows.

SEQUENCE LISTING (28 sequences)

SEQ ID NO: 1 - protein, 194 aa, Human Ssu72 protein sequence
MPSSPLRVAVVCSSNQNRSMEAHNILSKRGFSVRSFGTGTHVKLPGPAPDKPNVYDFKTTYDQMYNDLLRKDKELYTQNGILHMLDRNKRIKPRPERFQNCKDLFDLILTCEERVYDQVVEDLNSREQETCQPVHVVNVDIQDNHEEATLGAFLICELCQCIQHTEDMENEIDELLQEFEEKSGRTFLHTVCFY

SEQ ID NO: 2 - DNA, 585 bp, Human Ssu72 gene sequence
atgccgtcgtccccgctgcgggtggcggtggtgtgctcgagcaaccagaaccggagcatggaggcgcacaacatcctcagcaaacggggattcagcgtccgatcctttggaacagggactcacgtgaagcttccaggaccagctcccgacaagcccaatgtttatgatttcaaaaccacatatgaccagatgtacaatgatcttcttaggaaagacaaagaactctatacacagaatgggattttacatatgctggacagaaataagagaatcaagccccggccagaaagattccagaactgcaaagacctgtttgatctgatcctcacttgcgaagagagagtgtatgaccaggtggtggaagatctgaattccagagaacaggagacctgccagcctgtgcacgtggtcaatgtggacatccaggacaaccacgaggaggccaccctgggggcgtttctcatctgtgagctctgccagtgtatccagcacacggaagacatggagaacgagatcgacgagctgctgcaggagttcgaggagaagagtggccgcacctttctgcacaccgtctgcttctactga

SEQ ID NO: 3 - DNA, 5989 bp, pCMV. HA-Ssu72 plasmid
gacggatcgggagatctcccgatcccctatggtgcactctcagtacaatctgctctgatgccgcatagttaagccagtatctgctccctgcttgtgtgttggaggtcgctgagtagtgcgcgagcaaaatttaagctacaacaaggcaaggcttgaccgacaattgcatgaagaatctgcttagggttaggcgttttgcgctgcttcgcgatgtacgggccagatatacgcgttgacattgattattgactagttattaatagtaatcaattacggggtcattagttcatagcccatatatggagttccgcgttacataacttacggtaaatggcccgcctggctgaccgcccaacgacccccgcccattgacgtcaataatgacgtatgttcccatagtaacgccaatagggactttccattgacgtcaatgggtggagtatttacggtaaactgcccacttggcagtacatcaagtgtatcatatgccaagtacgccccctattgacgtcaatgacggtaaatggcccgcctggcattatgcccagtacatgaccttatgggactttcctacttggcagtacatctacgtattagtcatcgctattaccatggtgatgcggttttggcagtacatcaatgggcgtggatagcggtttgactcacggggatttccaagtctccaccccattgacgtcaatgggagtttgttttggcaccaaaatcaacgggactttccaaaatgtcgtaacaactccgccccattgacgcaaatgggcggtaggcgtgtacggtgggaggtctatataagcagagctctctggctaactagagaacccactgcttactggcttatcgaaattaatacgactcactatagggagacccagcttaccatggcctacccctacgacgtgcccgactacgcctccctcggatccatgccgtcgtccccgctgcgggtggcggtggtgtgctcgagcaaccagaaccggagcatggaggcgcacaacatcctcagcaaacggggattcagcgtccgatcctttggaacagggactcacgtgaagcttccaggaccagctcccgacaagcccaatgtttatgatttcaaaaccacatatgaccagatgtacaatgatcttcttaggaaagacaaagaactctatacacagaatgggattttacatatgctggacagaaataagagaatcaagccccggccagaaagattccagaactgcaaagacctgtttgatctgatcctcacttgcgaagagagagtgtatgaccaggtggtggaagatctgaattccagagaacaggagacctgccagcctgtgcacgtggtcaatgtggacatccaggacaaccacgaggaggccaccctgggggcgtttctcatctgtgagctctgccagtgtatccagcacacggaagacatggagaacgagatcgacgagctgctgcaggagttcgaggagaagagtggccgcacctttctgcacaccgtctgcttctactgatctagagggccctattctatagtgtcacctaaatgctagagctcgctgatcagcctcgactgtgccttctagttgccagccatctgttgtttgcccctcccccgtgccttccttgaccctggaaggtgccactcccactgtcctttcctaataaaatgaggaaattgcatcgcattgtctgagtaggtgtcattctattctggggggtggggtggggcaggacagcaagggggaggattgggaagacaatagcaggcatgctggggatgcggtgggctctatggcttctgaggcggaaagaaccagctggggctctagggggtatccccacgcgccctgtagcggcgcattaagcgcggcgggtgtggtggttacgcgcagcgtgaccgctacacttgccagcgccctagcgcccgctcctttcgctttcttcccttcctttctcgccacgttcgccggctttccccgtcaagctctaaatcgggggctccctttagggttccgatttagtgctttacggcacctcgaccccaaaaaacttgattagggtgatggttcacgtagtgggccatcgccctgatagacggtttttcgccctttgacgttggagtccacgttctttaatagtggactcttgttccaaactggaacaacactcaaccctatctcggtctattcttttgatttataagggattttgccgatttcggcctattggttaaaaaatgagctgatttaacaaaaatttaacgcgaattaattctgtggaatgtgtgtcagttagggtgtggaaagtccccaggctccccagcaggcagaagtatgcaaagcatgcatctcaattagtcagcaaccaggtgtggaaagtccccaggctccccagcaggcagaagtatgcaaagcatgcatctcaattagtcagcaaccatagtcccgcccctaactccgcccatcccgcccctaactccgcccagttccgcccattctccgccccatggctgactaattttttttatttatgcagaggccgaggccgcctctgcctctgagctattccagaagtagtgaggaggcttttttggaggcctaggcttttgcaaaaagctcccgggagcttgtatatccattttcggatctgatcaagagacaggatgaggatcgtttcgcatgattgaacaagatggattgcacgcaggttctccggccgcttgggtggagaggctattcggctatgactgggcacaacagacaatcggctgctctgatgccgccgtgttccggctgtcagcgcaggggcgcccggttctttttgtcaagaccgacctgtccggtgccctgaatgaactgcaggacgaggcagcgcggctatcgtggctggccacgacgggcgttccttgcgcagctgtgctcgacgttgtcactgaagcgggaagggactggctgctattgggcgaagtgccggggcaggatctcctgtcatctcaccttgctcctgccgagaaagtatccatcatggctgatgcaatgcggcggctgcatacgcttgatccggctacctgcccattcgaccaccaagcgaaacatcgcatcgagcgagcacgtactcggatggaagccggtcttgtcgatcaggatgatctggacgaagagcatcaggggctcgcgccagccgaactgttcgccaggctcaaggcgcgcatgcccgacggcgaggatctcgtcgtgacccatggcgatgcctgcttgccgaatatcatggtggaaaatggccgcttttctggattcatcgactgtggccggctgggtgtggcggaccgctatcaggacatagcgttggctacccgtgatattgctgaagagcttggcggcgaatgggctgaccgcttcctcgtgctttacggtatcgccgctcccgattcgcagcgcatcgccttctatcgccttcttgacgagttcttctgagcgggactctggggttcgaaatgaccgaccaagcgacgcccaacctgccatcacgagatttcgattccaccgccgccttctatgaaaggttgggcttcggaatcgttttccgggacgccggctggatgatcctccagcgcggggatctcatgctggagttcttcgcccaccccaacttgtttattgcagcttataatggttacaaataaagcaatagcatcacaaatttcacaaataaagcatttttttcactgcattctagttgtggtttgtccaaactcatcaatgtatcttatcatgtctgtataccgtcgacctctagctagagcttggcgtaatcatggtcatagctgtttcctgtgtgaaattgttatccgctcacaattccacacaacatacgagccggaagcataaagtgtaaagcctggggtgcctaatgagtgagctaactcacattaattgcgttgcgctcactgcccgctttccagtcgggaaacctgtcgtgccagctgcattaatgaatcggccaacgcgcggggagaggcggtttgcgtattgggcgctcttccgcttcctcgctcactgactcgctgcgctcggtcgttcggctgcggcgagcggtatcagctcactcaaaggcggtaatacggttatccacagaatcaggggataacgcaggaaagaacatgtgagcaaaaggccagcaaaaggccaggaaccgtaaaaaggccgcgttgctggcgtttttccataggctccgcccccctgacgagcatcacaaaaatcgacgctcaagtcagaggtggcgaaacccgacaggactataaagataccaggcgtttccccctggaagctccctcgtgcgctctcctgttccgaccctgccgcttaccggatacctgtccgcctttctcccttcgggaagcgtggcgctttctcatagctcacgctgtaggtatctcagttcggtgtaggtcgttcgctccaagctgggctgtgtgcacgaaccccccgttcagcccgaccgctgcgccttatccggtaactatcgtcttgagtccaacccggtaagacacgacttatcgccactggcagcagccactggtaacaggattagcagagcgaggtatgtaggcggtgctacagagttcttgaagtggtggcctaactacggctacactagaagaacagtatttggtatctgcgctctgctgaagccagttaccttcggaaaaagagttggtagctcttgatccggcaaacaaaccaccgctggtagcggtggtttttttgtttgcaagcagcagattacgcgcagaaaaaaaggatctcaagaagatcctttgatcttttctacggggtctgacgctcagtggaacgaaaactcacgttaagggattttggtcatgagattatcaaaaaggatcttcacctagatccttttaaattaaaaatgaagttttaaatcaatctaaagtatatatgagtaaacttggtctgacagttaccaatgcttaatcagtgaggcacctatctcagcgatctgtctatttcgttcatccatagttgcctgactccccgtcgtgtagataactacgatacgggagggcttaccatctggccccagtgctgcaatgataccgcgagacccacgctcaccggctccagatttatcagcaataaaccagccagccggaagggccgagcgcagaagtggtcctgcaactttatccgcctccatccagtctattaattgttgccgggaagctagagtaagtagttcgccagttaatagtttgcgcaacgttgttgccattgctacaggcatcgtggtgtcacgctcgtcgtttggtatggcttcattcagctccggttcccaacgatcaaggcgagttacatgatcccccatgttgtgcaaaaaagcggttagctccttcggtcctccgatcgttgtcagaagtaagttggccgcagtgttatcactcatggttatggcagcactgcataattctcttactgtcatgccatccgtaagatgcttttctgtgactggtgagtactcaaccaagtcattctgagaatagtgtatgcggcgaccgagttgctcttgcccggcgtcaatacgggataataccgcgccacatagcagaactttaaaagtgctcatcattggaaaacgttcttcggggcgaaaactctcaaggatcttaccgctgttgagatccagttcgatgtaacccactcgtgcacccaactgatcttcagcatcttttactttcaccagcgtttctgggtgagcaaaaacaggaaggcaaaatgccgcaaaaaagggaataagggcgacacggaaatgttgaatactcatactcttcctttttcaatattattgaagcatttatcagggttattgtctcatgagcggatacatatttgaatgtatttagaaaaataaacaaataggggttccgcgcacatttccccgaaaagtgccacctgacgtc

SEQ ID NO: 4 - DNA, 6456 bp, AAV8. TBG. HA-Ssu72
ctgcgcgctcgctcgctcactgaggccgcccgggcaaagcccgggcgtcgggcgacctttggtcgcccggcctcagtgagcgagcgagcgcgcagagagggagtggccaactccatcactaggggttccttgtagttaatgattaacccgccatgctacttatctaccagggtaatggggatcctctagaactatagctagaattcgcccttaagctagcaggttaatttttaaaaagcagtcaaaagtccaagtggcccttggcagcatttactctctctgtttgctctggttaataatctcaggagcacaaacattccagatccaggttaatttttaaaaagcagtcaaaagtccaagtggcccttggcagcatttactctctctgtttgctctggttaataatctcaggagcacaaacattccagatccggcgcgccagggctggaagctacctttgacatcatttcctctgcgaatgcatgtataatttctacagaacctattagaaaggatcacccagcctctgcttttgtacaactttcccttaaaaaactgccaattccactgctgtttggcccaatagtgagaactttttcctgctgcctcttggtgcttttgcctatggcccctattctgcctgctgaagacactcttgccagcatggacttaaacccctccagctctgacaatcctctttctcttttgttttacatgaagggtctggcagccaaagcaatcactcaaagttcaaaccttatcattttttgctttgttcctcttggccttggttttgtacatcagctttgaaaataccatcccagggttaatgctggggttaatttataactaagagtgctctagttttgcaatacaggacatgctataaaaatggaaagatgttgctttctgagagacagctttattgcggtagtttatcacagttaaattgctaacgcagtcagtgcttctgacacaacagtctcgaacttaagctgcagaagttggtcgtgaggcactgggcaggtaagtatcaaggttacaagacaggtttaaggagaccaatagaaactgggcttgtcgagacagagaagactcttgcgtttctgataggcacctattggtcttactgacatccactttgcctttctctccacaggtgtccactcccagttcaattacagctcttaaggctagagtacttaatacgactcactataggctagcaccatggaattcttttacccatacgatgttcctgactatgcgggctatccctatgacgtcccggactatgcaggatccatgccgtcgtccccgctgcgggtggcggtggtgtgctcgagcaaccagaaccggagcatggaggcgcacaacatcctcagcaaacggggattcagcgtccgatcctttggaacagggactcacgtgaagcttccaggaccagctcccgacaagcccaatgtttatgatttcaaaaccacatatgaccagatgtacaatgatcttcttaggaaagacaaagaactctatacacagaatgggattttacatatgctggacagaaataagagaatcaagccccggccagaaagattccagaactgcaaagacctgtttgatctgatcctcacttgcgaagagagagtgtatgaccaggtggtggaagatctgaattccagagaacaggagacctgccagcctgtgcacgtggtcaatgtggacatccaggacaaccacgaggaggccaccctgggggcgtttctcatctgtgagctctgccagtgtatccagcacacggaagacatggagaacgagatcgacgagctgctgcaggagttcgaggagaagagtggccgcacctttctgcacaccgtctgcttctactgaggtacccgctcgaggttaacgaattccgccccccccccccccccccccctctccctcccccccccctaacgttactggccgaagccgcttggaataaggccggtgtgcgtttgtctatatgttattttccaccatattgccgtcttttggcaatgtgagggcccggaaacctggccctgtcttcttgacgagcattcctaggggtctttcccctctcgccaaaggaatgcaaggtctgttgaatgtcgtgaaggaagcagttcctctggaagcttcttgaagacaaacaacgtctgtagcgaccctttgcaggcagcggaaccccccacctggcgacaggtgcctctgcggccaaaagccacgtgtataagatacacctgcaaaggcggcacaaccccagtgccacgttgtgagttggatagttgtggaaagagtcaaatggctctcctcaagcgtattcaacaaggggctgaaggatgcccagaaggtaccccattgtatgggatctgatctggggcctcggtgcacatgctttacatgtgtttagtcgaggttaaaaaaacgtctaggccccccgaaccacggggacgtggttttcctttgaaaaacacgatgataatatggccacaaccatggtgagcaagggcgaggagctgttcaccggggtggtgcccatcctggtcgagctggacggcgacgtaaacggccacaagttcagcgtgtctggcgagggcgagggcgatgccacctacggcaagctgaccctgaagttcatctgcaccaccggcaagctgcccgtgccctggcccaccctcgtgaccaccctgacctacggcgtgcagtgcttcagccgctaccccgaccacatgaagcagcacgacttcttcaagtccgccatgcccgaaggctacgtccaggagcgcaccatcttcttcaaggacgacggcaactacaagacccgcgccgaggtgaagttcgagggcgacaccctggtgaaccgcatcgagctgaagggcatcgacttcaaggaggacggcaacatcctggggcacaagctggagtacaactacaacagccacaacgtctatatcatggccgacaagcagaagaacggcatcaaggcgaacttcaagatccgccacaacatcgaggacggcagcgtgcagctcgccgaccactaccagcagaacacccccatcggcgacggccccgtgctgctgcccgacaaccactacctgagcacccagtccgccctgagcaaagaccccaacgagaagcgcgatcacatggtcctgctggagttcgtgaccgccgccgggatcactctcggcatggacgagctgtacaagtaagtcgacccgggcggcctcgaggacggggtgaactacgcctgaggatccgatctttttccctctgccaaaaattatggggacatcatgaagccccttgagcatctgacttctggctaataaaggaaatttattttcattgcaatagtgtgttggaattttttgtgtctctcactcggaagcaattcgttgatctgaatttcgaccacccataatacccattaccctggtagataagtagcatggcgggttaatcattaactacaaggaacccctagtgatggagttggccactccctctctgcgcgctcgctcgctcactgaggccgggcgaccaaaggtcgcccgacgcccgggctttgcccgggcggcctcagtgagcgagcgagcgcgcagccttaattaacctaattcactggccgtcgttttacaacgtcgtgactgggaaaaccctggcgttacccaacttaatcgccttgcagcacatccccctttcgccagctggcgtaatagcgaagaggcccgcaccgatcgcccttcccaacagttgcgcagcctgaatggcgaatgggacgcgccctgtagcggcgcattaagcgcggcgggtgtggtggttacgcgcagcgtgaccgctacacttgccagcgccctagcgcccgctcctttcgctttcttcccttcctttctcgccacgttcgccggctttccccgtcaagctctaaatcgggggctccctttagggttccgatttagtgctttacggcacctcgaccccaaaaaacttgattagggtgatggttcacgtagtgggccatcgccctgatagacggtttttcgccctttgacgttggagtccacgttctttaatagtggactcttgttccaaactggaacaacactcaaccctatctcggtctattcttttgatttataagggattttgccgatttcggcctattggttaaaaaatgagctgatttaacaaaaatttaacgcgaattttaacaaaatattaacgcttacaatttaggtggcacttttcggggaaatgtgcgcggaacccctatttgtttatttttctaaatacattcaaatatgtatccgctcatgagacaataaccctgataaatgcttcaataatattgaaaaaggaagagtatgagtattcaacatttccgtgtcgcccttattcccttttttgcggcattttgccttcctgtttttgctcacccagaaacgctggtgaaagtaaaagatgctgaagatcagttgggtgcacgagtgggttacatcgaactggatctcaacagcggtaagatccttgagagttttcgccccgaagaacgttttccaatgatgagcacttttaaagttctgctatgtggcgcggtattatcccgtattgacgccgggcaagagcaactcggtcgccgcatacactattctcagaatgacttggttgagtactcaccagtcacagaaaagcatcttacggatggcatgacagtaagagaattatgcagtgctgccataaccatgagtgataacactgcggccaacttacttctgacaacgatcggaggaccgaaggagctaaccgcttttttgcacaacatgggggatcatgtaactcgccttgatcgttgggaaccggagctgaatgaagccataccaaacgacgagcgtgacaccacgatgcctgtagcaatggcaacaacgttgcgcaaactattaactggcgaactacttactctagcttcccggcaacaattaatagactggatggaggcggataaagttgcaggaccacttctgcgctcggcccttccggctggctggtttattgctgataaatctggagccggtgagcgtgggtctcgcggtatcattgcagcactggggccagatggtaagccctcccgtatcgtagttatctacacgacggggagtcaggcaactatggatgaacgaaatagacagatcgctgagataggtgcctcactgattaagcattggtaactgtcagaccaagtttactcatatatactttagattgatttaaaacttcatttttaatttaaaaggatctaggtgaagatcctttttgataatctcatgaccaaaatcccttaacgtgagttttcgttccactgagcgtcagaccccgtagaaaagatcaaaggatcttcttgagatcctttttttctgcgcgtaatctgctgcttgcaaacaaaaaaaccaccgctaccagcggtggtttgtttgccggatcaagagctaccaactctttttccgaaggtaactggcttcagcagagcgcagataccaaatactgttcttctagtgtagccgtagttaggccaccacttcaagaactctgtagcaccgcctacatacctcgctctgctaatcctgttaccagtggctgctgccagtggcgataagtcgtgtcttaccgggttggactcaagacgatagttaccggataaggcgcagcggtcgggctgaacggggggttcgtgcacacagcccagcttggagcgaacgacctacaccgaactgagatacctacagcgtgagctatgagaaagcgccacgcttcccgaagggagaaaggcggacaggtatccggtaagcggcagggtcggaacaggagagcgcacgagggagcttccagggggaaacgcctggtatctttatagtcctgtcgggtttcgccacctctgacttgagcgtcgatttttgtgatgctcgtcaggggggcggagcctatggaaaaacgccagcaacgcggcctttttacggttcctggccttttgctggccttttgctcacatgttctttcctgcgttatcccctgattctgtggataaccgtattaccgcctttgagtgagctgataccgctcgccgcagccgaacgaccgagcgcagcgagtcagtgagcgaggaagcggaagagcgcccaatacgcaaaccgcctctccccgcgcgttggccgattcattaatgcagctggcacgacaggtttcccgactggaaagcgggcagtgagcgcaacgcaattaatgtgagttagctcactcattaggcaccccaggctttacactttatgcttccggctcgtatgttgtgtggaattgtgagcggataacaatttcacacaggaaacagctatgaccatgattacgccagatttaattaaggccttaattagg

SEQ ID NO: 5 - DNA, 19 bp, Artificial Sequence
  TGF-beta forward primer
caccggagagccctggata

SEQ ID NO: 6 - DNA, 19 bp, Artificial Sequence
  TGF-beta reverse primer
caccggagagccctggata

SEQ ID NO: 7 - DNA, 25 bp, Artificial Sequence
  Colla1 forward primer
gggtctagacatgttcagctttgtg

SEQ ID NO: 8 - DNA, 22 bp, Artificial Sequence
  Colla1 reverse primer
acccttaggccattgtgtatgc

SEQ ID NO: 9 - DNA, 20 bp, Artificial Sequence
  Fasn forward primer
attgcatcaagcaagtgcag

SEQ ID NO: 10 - DNA, 19 bp, Artificial Sequence
  Fasn reverse primer
gagccgtcaaacaggaaag

SEQ ID NO: 11 - DNA, 19 bp, Artificial Sequence
  Srebp1c forward primer
ggcttgtcctttgggaagc

SEQ ID NO: 12 - DNA, 18 bp, Artificial Sequence
  Srebp1c reverse primer
cgcctatgctggtgcaca

SEQ ID NO: 13 - DNA, 20 bp, Artificial Sequence
  ACC1 forward primer
ccaggccatgttgagacgct

SEQ ID NO: 14 - DNA, 20 bp, Artificial Sequence
  ACC1 reverse primer
ccagccagcctcttgactat

SEQ ID NO: 15 - DNA, 22 bp, Artificial Sequence
  PPARa forward primer
ggatgtcacacaatgcaattcg

SEQ ID NO: 16 - DNA, 22 bp, Artificial Sequence
  PPARa reverse primer
tcacagaacggcttcctcaggt

SEQ ID NO: 17 - DNA, 19 bp, Artificial Sequence
  Pgcla forward primer
ccctgccattgttaagacc

SEQ ID NO: 18 - DNA, 19 bp, Artificial Sequence
  Pgcla reverse primer
tgctgctgttcctgttttc

SEQ ID NO: 19 - DNA, 20 bp, Artificial Sequence
  Col3a1 forward primer
tacacctgctcctgtgcttc

SEQ ID NO: 20 - DNA, 20 bp, Artificial Sequence
  Col3a1 reverse primer
cattcctcccactccagact

SEQ ID NO: 21 - DNA, 19 bp, Artificial Sequence
  MMP12 forward primer
accagagccacactatccc

SEQ ID NO: 22 - DNA, 20 bp, Artificial Sequence
  MMP12 reverse primer
ctcctgcctcacatcatacc

SEQ ID NO: 23 - DNA, 19 bp, Artificial Sequence
  MMP13 forward primer
ctggcacacgcttttcctc

SEQ ID NO: 24 - DNA, 22 bp, Artificial Sequence
  MMP13 reverse primer
atgggcagcaacaataaacaag

SEQ ID NO: 25 - DNA, 20 bp, Artificial Sequence
  SMA forward primer
ctgacagaggcaccactgaa

SEQ ID NO: 26 - DNA, 20 bp, Artificial Sequence
  SMA reverse primer
catctccagagtccagcaca

SEQ ID NO: 27 - DNA, 22 bp, Artificial Sequence
  Timp forward primer
ctcaaagacctatagtgctggc

SEQ ID NO: 28 - DNA, 20 bp, Artificial Sequence
  Timp reverse primer
caaagtgacggctctggtag